European Patent Specification EP 3 455 240 B1, published January 1, 2025. Title: MUTATED IMMUNOGLOBULIN-BINDING POLYPEPTIDES. Applicant: GE Healthcare Bioprocess R&D AB. The sequence listing filed with the application follows.

SEQUENCE LISTING (95 sequences)

SEQ ID NO: 1 - protein, 51 aa, Staphylococcus aureus
AQQNAFYQVLNMPNLNADQRNGFIQSLKDDPSQSANVLGEAQKLNDSQAPK

SEQ ID NO: 2 - protein, 61 aa, Staphylococcus aureus
ADAQQNKFNKDQQSAFYEILNMPNLNEEQRNGFIQSLKDDPSQSTNVLGEAKKLNESQAPK

SEQ ID NO: 3 - protein, 58 aa, Staphylococcus aureus
ADNNFNKEQQNAFYEILNMPNLNEEQRNGFIQSLKDDPSQSANLLAEAKKLNESQAPK

SEQ ID NO: 4 - protein, 58 aa, Staphylococcus aureus [sequence omitted]

SEQ ID NO: 5 - protein, 58 aa, Staphylococcus aureus
ADNKFNKEQQNAFYEILHLPNLTEEQRNGFIQSLKDDPSVSKEILAEAKKLNDAQAPK

SEQ ID NO: 6 - protein, 58 aa, Escherichia coli [sequence omitted]

SEQ ID NO: 7 - protein, 58 aa, Escherichia coli [sequence omitted]

SEQ ID NO: 8 - protein, 58 aa, Escherichia coli
VDAKFDKEAQEAFYEILHLPNLTEEQRNAFIQSLKDDPSQSAALLAEAKKLNDAQAPK

SEQ ID NO: 9 - protein, 58 aa, Escherichia coli
VDAKFDKEAQEAFYEILHLPNLTEEQRAAFIQSLKDDPSQSAALLAEAKKLNDAQAPK

SEQ ID NO: 10 - protein, 58 aa, Escherichia coli
VDAKFDKEAQEAFYEILHLPNLTEEQRNAFIQSLKDDPSVSKEILAEAKKLNDAQAPK

SEQ ID NO: 11 - protein, 58 aa, Escherichia coli
VDAKFDKEAQEAFYEILHLPNLTEEQRNAFIQSLKDDPSVSKAILAEAKKLNDAQAPK

SEQ ID NO: 12 - protein, 58 aa, Escherichia coli
VDAKFDKEQQEAFYEILHLPNLTEEQRNAFIASLKDDPSQSANLLAEAKKLNDAQAPK

SEQ ID NO: 13 - protein, 58 aa, Escherichia coli
VDAKFDKEQQEAFYEILHLPNLTEEQRNAFIQSLKDDPSQSANLLAEAKKLNDAQAPK

SEQ ID NO: 14 - protein, 58 aa, Escherichia coli
VDAKFDKEQQEAFYEILHLPNLTEEQRNAFIESLKDDPSESANLLAEAKKLNDAQAPK

SEQ ID NO: 15 - protein, 58 aa, Escherichia coli
VDAKFDKEQQEAFYEILHLPNLTEEQRNAFIESLKDDPSQSANLLAEAKRLNDAQAPK

SEQ ID NO: 16 - protein, 58 aa, Escherichia coli
VDAKFDKEQQKAFYEILHLPNLTEEQRNAFIQSLKDDPSQSANLLAEAKKLNDAQAPK

SEQ ID NO: 17 - protein, 237 aa, Escherichia coli
AQGTVDAKFDKEAQEAFYEILHLPNLTEEQRNAFIQSLKDDPSQSAALLAEAKKLNDAQAPKVDAKFDKEAQEAFYEILHLPNLTEEQRNAFIQSLKDDPSQSAALLAEAKKLNDAQAPKVDAKFDKEAQEAFYEILHLPNLTEEQRNAFIQSLKDDPSQSAALLAEAKKLNDAQAPKVDAKFDKEAQEAFYEILHLPNLTEEQRNAFIQSLKDDPSQSAALLAEAKKLNDAQAPKC

SEQ ID NO: 18 - protein, 237 aa, Escherichia coli
AQGTVDAKFDKEAQEAFYEILHLPNLTEEQRAAFIQSLKDDPSQSAALLAEAKKLNDAQAPKVDAKFDKEAQEAFYEILHLPNLTEEQRAAFIQSLKDDPSQSAALLAEAKKLNDAQAPKVDAKFDKEAQEAFYEILHLPNLTEEQRAAFIQSLKDDPSQSAALLAEAKKLNDAQAPKVDAKFDKEAQEAFYEILHLPNLTEEQRAAFIQSLKDDPSQSAALLAEAKKLNDAQAPKC

SEQ ID NO: 19 - protein, 237 aa, Escherichia coli
AQGTVDAKFDKEAQEAFYEILHLPNLTEEQRNAFIQSLKDDPSVSKEILAEAKKLNDAQAPKVDAKFDKEAQEAFYEILHLPNLTEEQRNAFIQSLKDDPSVSKEILAEAKKLNDAQAPKVDAKFDKEAQEAFYEILHLPNLTEEQRNAFIQSLKDDPSVSKEILAEAKKLNDAQAPKVDAKFDKEAQEAFYEILHLPNLTEEQRNAFIQSLKDDPSVSKEILAEAKKLNDAQAPKC

SEQ ID NO: 20 - protein, 237 aa, Escherichia coli
AQGTVDAKFDKEAQEAFYEILHLPNLTEEQRNAFIQSLKDDPSVSKAILAEAKKLNDAQAPKVDAKFDKEAQEAFYEILHLPNLTEEQRNAFIQSLKDDPSVSKAILAEAKKLNDAQAPKVDAKFDKEAQEAFYEILHLPNLTEEQRNAFIQSLKDDPSVSKAILAEAKKLNDAQAPKVDAKFDKEAQEAFYEILHLPNLTEEQRNAFIQSLKDDPSVSKAILAEAKKLNDAQAPKC

SEQ ID NO: 21 - protein, 237 aa, Escherichia coli
AQGTVDAKFDKEQQNAFYEILHLPNLTEEQRNAFIQSLKDDPSQSANLLAEAKKLNDAQAPKVDAKFDKEQQNAFYEILHLPNLTEEQRNAFIQSLKDDPSQSANLLAEAKKLNDAQAPKVDAKFDKEQQNAFYEILHLPNLTEEQRNAFIQSLKDDPSQSANLLAEAKKLNDAQAPKVDAKFDKEQQNAFYEILHLPNLTEEQRNAFIQSLKDDPSQSANLLAEAKKLNDAQAPKC

SEQ ID NO: 22 - protein, 58 aa, Staphylococcus aureus
ADNNFNKEQQNAFYEILNMPNLNEEQRNGFIQSLKDDPSQSANLLSEAKKLNESQAPK

SEQ ID NO: 23 - protein, 58 aa, Escherichia coli
VDAKFDKEQQKAFYEILKLPNLTEEQRNAFIQKLKDEPSQSRAILAEAKRYNDAQAPK

SEQ ID NO: 24 - protein, 58 aa, Escherichia coli
VDAKFDKEAQEAFYEILHLPNLTEEQRAAFIQSLKDDPSVSKAILAEAKKLNDAQAPK

SEQ ID NO: 25 - protein, 58 aa, Escherichia coli
VDAKFDKEAQKAFYEILKLPNLTEEQRAAFIQKLKDEPSQSRAILAEAKRYNDAQAPK

SEQ ID NO: 26 - protein, 58 aa, Escherichia coli
VDAKFDKEQQKAFYEILKLPNLTEEQRNAFIQSLKDEPSQSRAILAEAKKLNDAQAPK

SEQ ID NO: 27 - protein, 58 aa, Escherichia coli
VDAKFDKEAQKAFYEILKLPNLTEEQRNAFIQSLKDEPSQSRAILAEAKKLNDAQAPK

SEQ ID NO: 28 - protein, 58 aa, Escherichia coli
VDAKFDKEAQKAFYEILKLPNLTEEQRNAFIQSLKDEPSQSRAILAEAKRLNDAQAPK

SEQ ID NO: 29 - protein, 58 aa, Escherichia coli
VDAKFDKEAQKAFYEILKLPNLTEEQRNAFIQSLKDEPSQSRNLLAEAKKLNDAQAPK

SEQ ID NO: 30 - protein, 237 aa, Escherichia coli
AQGTVDAKFDKEQQKAFYEILKLPNLTEEQRNAFIQKLKDEPSQSRAILAEAKRYNDAQAPKVDAKFDKEQQKAFYEILKLPNLTEEQRNAFIQKLKDEPSQSRAILAEAKRYNDAQAPKVDAKFDKEQQKAFYEILKLPNLTEEQRNAFIQKLKDEPSQSRAILAEAKRYNDAQAPKVDAKFDKEQQKAFYEILKLPNLTEEQRNAFIQKLKDEPSQSRAILAEAKRYNDAQAPKC

SEQ ID NO: 31 - protein, 237 aa, Escherichia coli
AQGTVDAKFDKEAQKAFYEILKLPNLTEEQRNAFIQSLKDEPSQSRNLLAEAKKLNDAQAPKVDAKFDKEAQKAFYEILKLPNLTEEQRNAFIQSLKDEPSQSRNLLAEAKKLNDAQAPKVDAKFDKEAQKAFYEILKLPNLTEEQRNAFIQSLKDEPSQSRNLLAEAKKLNDAQAPKVDAKFDKEAQKAFYEILKLPNLTEEQRNAFIQSLKDEPSQSRNLLAEAKKLNDAQAPKC

SEQ ID NO: 32 - protein, 237 aa, Escherichia coli
AQGTVDAKFDKEAQEAFYEILHLPNLTEEQRAAFIQSLKDDPSVSKAILAEAKKLNDAQAPKVDAKFDKEAQEAFYEILHLPNLTEEQRAAFIQSLKDDPSVSKAILAEAKKLNDAQAPKVDAKFDKEAQEAFYEILHLPNLTEEQRAAFIQSLKDDPSVSKAILAEAKKLNDAQAPKVDAKFDKEAQEAFYEILHLPNLTEEQRAAFIQSLKDDPSVSKAILAEAKKLNDAQAPKC

SEQ ID NO: 33 - protein, 353 aa, Escherichia coli
AQGTVDAKFDKEAQEAFYEILHLPNLTEEQRNAFIQSLKDDPSVSKAILAEAKKLNDAQAPKVDAKFDKEAQEAFYEILHLPNLTEEQRNAFIQSLKDDPSVSKAILAEAKKLNDAQAPKVDAKFDKEAQEAFYEILHLPNLTEEQRNAFIQSLKDDPSVSKAILAEAKKLNDAQAPKVDAKFDKEAQEAFYEILHLPNLTEEQRNAFIQSLKDDPSVSKAILAEAKKLNDAQAPKVDAKFDKEAQEAFYEILHLPNLTEEQRNAFIQSLKDDPSVSKAILAEAKKLNDAQAPKVDAKFDKEAQEAFYEILHLPNLTEEQRNAFIQSLKDDPSVSKAILAEAKKLNDAQAPKC

SEQ ID NO: 34 - protein, 237 aa, Escherichia coli
AQGTVDAKFDKEAQEAFYEILHLPNLTEEQRNAFIQSLKDEPSVSKAILAEAKKLNDAQAPKVDAKFDKEAQEAFYEILHLPNLTEEQRNAFIQSLKDEPSVSKAILAEAKKLNDAQAPKVDAKFDKEAQEAFYEILHLPNLTEEQRNAFIQSLKDEPSVSKAILAEAKKLNDAQAPKVDAKFDKEAQEAFYEILHLPNLTEEQRNAFIQSLKDEPSVSKAILAEAKKLNDAQAPKC

SEQ ID NO: 35 - protein, 237 aa, Escherichia coli
AQGTVDAKFDKEAQEAFYEILHLPNLTEEQRNAFIQSLKDEPSVSRAILAEAKKLNDAQAPKVDAKFDKEAQEAFYEILHLPNLTEEQRNAFIQSLKDEPSVSRAILAEAKKLNDAQAPKVDAKFDKEAQEAFYEILHLPNLTEEQRNAFIQSLKDEPSVSRAILAEAKKLNDAQAPKVDAKFDKEAQEAFYEILHLPNLTEEQRNAFIQSLKDEPSVSRAILAEAKKLNDAQAPKC

SEQ ID NO: 36 - protein, 58 aa, Escherichia coli
ADNKFNKEAQEAFYEILHLPNLNEEQRNGFIQSLKDDPSVSKAILAEAKKLNDAQAPK

SEQ ID NO: 37 - protein, 58 aa, Escherichia coli
ADNKFNKEAQEAFYEILHLPNLTEEQRNGFIQSLKDDPSVSKAILAEAKKLNDAQAPK

SEQ ID NO: 38 - protein, 58 aa, Escherichia coli
VDAKFDKEQQYAFYEILHLPNLTEEQRNAFIQSLKDDPSQSANLLAEAKKLNDAQAPK

SEQ ID NO: 39 - protein, 58 aa, Escherichia coli
VDAKFDKEQQTAFYEILHLPNLTEEQRNAFIQSLKDDPSQSANLLAEAKKLNDAQAPK

SEQ ID NO: 40 - protein, 58 aa, Escherichia coli
VDAKFDKEQQFAFYEILHLPNLTEEQRNAFIQSLKDDPSQSANLLAEAKKLNDAQAPK

SEQ ID NO: 41 - protein, 58 aa, Escherichia coli
VDAKFDKEQQLAFYEILHLPNLTEEQRNAFIQSLKDDPSQSANLLAEAKKLNDAQAPK

SEQ ID NO: 42 - protein, 58 aa, Escherichia coli
VDAKFDKEQQWAFYEILHLPNLTEEQRNAFIQSLKDDPSQSANLLAEAKKLNDAQAPK

SEQ ID NO: 43 - protein, 58 aa, Escherichia coli
VDAKFDKEQQIAFYEILHLPNLTEEQRNAFIQSLKDDPSQSANLLAEAKKLNDAQAPK

SEQ ID NO: 44 - protein, 58 aa, Escherichia coli
VDAKFDKEQQMAFYEILHLPNLTEEQRNAFIQSLKDDPSQSANLLAEAKKLNDAQAPK

SEQ ID NO: 45 - protein, 58 aa, Escherichia coli
VDAKFDKEQQVAFYEILHLPNLTEEQRNAFIQSLKDDPSQSANLLAEAKKLNDAQAPK

SEQ ID NO: 46 - protein, 58 aa, Escherichia coli
VDAKFDKEQQAAFYEILHLPNLTEEQRNAFIQSLKDDPSQSANLLAEAKKLNDAQAPK

SEQ ID NO: 47 - protein, 58 aa, Escherichia coli
VDAKFDKEQQHAFYEILHLPNLTEEQRNAFIQSLKDDPSQSANLLAEAKKLNDAQAPK

SEQ ID NO: 48 - protein, 58 aa, Escherichia coli
VDAKFDKEQQRAFYEILHLPNLTEEQRNAFIQSLKDDPSQSANLLAEAKKLNDAQAPK

SEQ ID NO: 49 - protein, 58 aa, Escherichia coli
VDAKFDKEAQEAFYEILHLPNLTEEQRNAFIQSLKDEPSVSKAILAEAKKLNDAQAPK

SEQ ID NO: 50 - protein, 58 aa, Escherichia coli
VDAKFDKEAQEAFYEILHLPNLTEEQRNAFIQSLKDEPSVSRAILAEAKKLNDAQAPK

SEQ ID NO: 51 - protein, 47 aa, Escherichia coli
QQNAFYEILHLPNLTEEQRNAFIQSLKDDPSQSANLLAEAKKLNDAQ

SEQ ID NO: 52 - protein, 47 aa, Staphylococcus aureus
QQNAFYEILHLPNLTEEQRNGFIQSLKDDPSVSKEILAEAKKLNDAQ

SEQ ID NO: 53 - protein, 47 aa, Escherichia coli
  misc_feature (1)..(1): Xaa can be any naturally occurring amino acid
  misc_feature (3)..(3): Xaa can be any naturally occurring amino acid
  misc_feature (10)..(10): Xaa can be any naturally occurring amino acid
  misc_feature (20)..(21): Xaa can be any naturally occurring amino acid
  misc_feature (24)..(25): Xaa can be any naturally occurring amino acid
  misc_feature (29)..(29): Xaa can be any naturally occurring amino acid
  misc_feature (32)..(32): Xaa can be any naturally occurring amino acid
  misc_feature (34)..(36): Xaa can be any naturally occurring amino acid
  misc_feature (42)..(43): Xaa can be any naturally occurring amino acid
  misc_feature (45)..(45): Xaa can be any naturally occurring amino acid
XQXAFYEILXLPNLTEEQRXXFIXXLKDXPSXSXXXLAEAKXXNXAQ

SEQ ID NO: 54 - protein, 58 aa, Escherichia coli
VDAKFDKEAQEAFYEILHLPNLTEEQRNGFIQSLKDDPSVSKAILAEAKKLNDAQAPK

SEQ ID NO: 55 - protein, 58 aa, Escherichia coli
VDAKFDKEAQEAFYEILHLPNLTEEQRNSFIQSLKDDPSVSKAILAEAKKLNDAQAPK

SEQ ID NO: 56 - protein, 58 aa, Escherichia coli
VDAKFDKEAQEAFYEILHLPNLTEEQRNYFIQSLKDDPSVSKAILAEAKKLNDAQAPK

SEQ ID NO: 57 - protein, 58 aa, Escherichia coli
VDAKFDKEAQEAFYEILHLPNLTEEQRNQFIQSLKDDPSVSKAILAEAKKLNDAQAPK

SEQ ID NO: 58 - protein, 58 aa, Escherichia coli
VDAKFDKEAQEAFYEILHLPNLTEEQRNTFIQSLKDDPSVSKAILAEAKKLNDAQAPK

SEQ ID NO: 59 - protein, 58 aa, Escherichia coli
VDAKFDKEAQEAFYEILHLPNLTEEQRNNFIQSLKDDPSVSKAILAEAKKLNDAQAPK

SEQ ID NO: 60 - protein, 58 aa, Escherichia coli
VDAKFDKEAQEAFYEILHLPNLTEEQRNFFIQSLKDDPSVSKAILAEAKKLNDAQAPK

SEQ ID NO: 61 - protein, 58 aa, Escherichia coli
VDAKFDKEAQEAFYEILHLPNLTEEQRNLFIQSLKDDPSVSKAILAEAKKLNDAQAPK

SEQ ID NO: 62 - protein, 58 aa, Escherichia coli
VDAKFDKEAQEAFYEILHLPNLTEEQRNWFIQSLKDDPSVSKAILAEAKKLNDAQAPK

SEQ ID NO: 63 - protein, 58 aa, Escherichia coli
VDAKFDKEAQEAFYEILHLPNLTEEQRNIFIQSLKDDPSVSKAILAEAKKLNDAQAPK

SEQ ID NO: 64 - protein, 58 aa, Escherichia coli
VDAKFDKEAQEAFYEILHLPNLTEEQRNMFIQSLKDDPSVSKAILAEAKKLNDAQAPK

SEQ ID NO: 65 - protein, 58 aa, Escherichia coli
VDAKFDKEAQEAFYEILHLPNLTEEQRNVFIQSLKDDPSVSKAILAEAKKLNDAQAPK

SEQ ID NO: 66 - protein, 58 aa, Escherichia coli
VDAKFDKEAQEAFYEILHLPNLTEEQRNDFIQSLKDDPSVSKAILAEAKKLNDAQAPK

SEQ ID NO: 67 - protein, 58 aa, Escherichia coli
VDAKFDKEAQEAFYEILHLPNLTEEQRNEFIQSLKDDPSVSKAILAEAKKLNDAQAPK

SEQ ID NO: 68 - protein, 58 aa, Escherichia coli
VDAKFDKEAQEAFYEILHLPNLTEEQRNHFIQSLKDDPSVSKAILAEAKKLNDAQAPK

SEQ ID NO: 69 - protein, 58 aa, Escherichia coli
VDAKFDKEAQEAFYEILHLPNLTEEQRNRFIQSLKDDPSVSKAILAEAKKLNDAQAPK

SEQ ID NO: 70 - protein, 58 aa, Escherichia coli
VDAKFDKEAQEAFYEILHLPNLTEEQRNKFIQSLKDDPSVSKAILAEAKKLNDAQAPK

SEQ ID NO: 71 - protein, 58 aa, Escherichia coli
VDAKFDKEAQEAFYEILHLPNLTEEQRNAFIQSLKDDPSVSKAILAEAKKLNFAQAPK

SEQ ID NO: 72 - protein, 58 aa, Escherichia coli
VDAKFDKEAQEAFYEILHLPNLTEEQRNAFIQSLKDDPSVSKAILAEAKKLNYAQAPK

SEQ ID NO: 73 - protein, 58 aa, Escherichia coli
VDAKFDKEAQEAFYEILHLPNLTEEQRNAFIQSLKDDPSVSKAILAEAKKLNWAQAPK

SEQ ID NO: 74 - protein, 58 aa, Escherichia coli
VDAKFDKEAQEAFYEILHLPNLTEEQRNAFIQSLKDDPSVSKAILAEAKKLNKAQAPK

SEQ ID NO: 75 - protein, 58 aa, Escherichia coli
VDAKFDKEAQEAFYEILHLPNLTEEQRNAFIQSLKDDPSVSKAILAEAKKLNRAQAPK

SEQ ID NO: 76 - protein, 57 aa, Escherichia coli
VDAKFDKEQEAFYEILHLPNLTEEQRNAFIQSLKDDPSVSKAILAEAKKLNDAQAPK

SEQ ID NO: 77 - protein, 57 aa, Escherichia coli
VDAKFDKEAQEAFYEILHLPNLTEEQRNAFIQSLKDDPSSKAILAEAKKLNDAQAPK

SEQ ID NO: 78 - protein, 57 aa, Escherichia coli
VDAKFDKEAQEAFYEILHLPNLTEEQRNAFIQSLKDDPSVSAILAEAKKLNDAQAPK

SEQ ID NO: 79 - protein, 57 aa, Escherichia coli
VDAKFDKEAQEAFYEILHLPNLTEEQRNAFIQSLKDDPSVSKILAEAKKLNDAQAPK

SEQ ID NO: 80 - protein, 114 aa, Escherichia coli
VDAKFDKEAQEAFYEILHLPNLTEEQRNAFIQSLKDDPSVSKAILAEAKKLNDAQAPKVFDKEAQEAFYEILHLPNLTEEQRNAFIQSLKDDPSVSKAILAEAKKLNDAQAPKC

SEQ ID NO: 81 - protein, 114 aa, Escherichia coli
VDAKFDKEAQEAFYEILHLPNLTEEQRNAFIQSLKDDPSVSKAILAEAKKLNDAQAPAKFDKEAQEAFYEILHLPNLTEEQRNAFIQSLKDDPSVSKAILAEAKKLNDAQAPKC

SEQ ID NO: 82 - protein, 114 aa, Escherichia coli; identical to SEQ ID NO: 81

SEQ ID NO: 83 - protein, 112 aa, Escherichia coli
VDAKFDKEAQEAFYEILHLPNLTEEQRNAFIQSLKDDPSVSKAILAEAKKLNDAQAPKVDAAQEAFYEILHLPNLTEEQRNAFIQSLKDDPSVSKAILAEAKKLNDAQAPKC

SEQ ID NO: 84 - protein, 114 aa, Escherichia coli
VDAKFDKEAQEAFYEILHLPNLTEEQRNAFIQSLKDDPSVSKAILAEAKKLNDAQVDAKFDKEAQEAFYEILHLPNLTEEQRNAFIQSLKDDPSVSKAILAEAKKLNDAQAPKC

SEQ ID NO: 85 - protein, 114 aa, Escherichia coli
VDAKFDKEAQEAFYEILHLPNLTEEQRNAFIQSLKDDPSVSKAILAEAKKLNDAQAPKKFDKEAQEAFYEILHLPNLTEEQRNAFIQSLKDDPSVSKAILAEAKKLNDAQAPKC

SEQ ID NO: 86 - protein, 109 aa, Escherichia coli
VDAKFDKEAQEAFYEILHLPNLTEEQRNAFIQSLKDDPSVSKAILAEAKKLNDAQAPKAQEAFYEILHLPNLTEEQRNAFIQSLKDDPSVSKAILAEAKKLNDAQAPKC

SEQ ID NO: 87 - protein, 121 aa, Escherichia coli
VDAKFDKEAQEAFYEILHLPNLTEEQRNAFIQSLKDDPSVSKAILAEAKKLNDAQAPKYEDGVDAKFDKEAQEAFYEILHLPNLTEEQRNAFIQSLKDDPSVSKAILAEAKKLNDAQAPKC

SEQ ID NO: 88 - protein, 117 aa, Escherichia coli
VDAKFDKEAQEAFYEILHLPNLTEEQRNAFIQSLKDDPSVSKAILAEAKKLNDAQAPKVDAKFDKEAQEAFYEILHLPNLTEEQRNAFIQSLKDDPSVSKAILAEAKKLNDAQAPKC

SEQ ID NO: 89 - protein, 55 aa, Escherichia coli
VFDKEAQEAFYEILHLPNLTEEQRNAFIQSLKDDPSVSKAILAEAKKLNDAQAPK

SEQ ID NO: 90 - protein, 55 aa, Escherichia coli
AKFDKEAQEAFYEILHLPNLTEEQRNAFIQSLKDDPSVSKAILAEAKKLNDAQAP

SEQ ID NO: 91 - protein, 53 aa, Escherichia coli
VDAAQEAFYEILHLPNLTEEQRNAFIQSLKDDPSVSKAILAEAKKLNDAQAPK

SEQ ID NO: 92 - protein, 55 aa, Escherichia coli
VDAKFDKEAQEAFYEILHLPNLTEEQRNAFIQSLKDDPSVSKAILAEAKKLNDAQ

SEQ ID NO: 93 - protein, 55 aa, Escherichia coli
KFDKEAQEAFYEILHLPNLTEEQRNAFIQSLKDDPSVSKAILAEAKKLNDAQAPK

SEQ ID NO: 94 - protein, 50 aa, Escherichia coli
AQEAFYEILHLPNLTEEQRNAFIQSLKDDPSVSKAILAEAKKLNDAQAPK

SEQ ID NO: 95 - protein, 62 aa, Escherichia coli
VDAKFDKEAQEAFYEILHLPNLTEEQRNAFIQSLKDDPSVSKAILAEAKKLNDAQAPKYEDG